European Patent Specification EP 4 003 415 B1, published September 11, 2024. Title: Inhibitors of CHI3L1 and their uses. Applicant: Humanitas Mirasole S.p.A. Humanitas University. The sequence listing filed with the application follows.

SEQUENCE LISTING (2 sequences)

SEQ ID NO: 1 - DNA, 1152 bp, Homo sapiens
atgggtgtgaaggcgtctcaaacaggctttgtggtcctggtgctgctccagtgctgctctgcatacaaactggtctgctactacaccagctggtcccagtaccgggaaggcgatgggagctgcttcccagatgcccttgaccgcttcctctgtacccacatcatctacagctttgccaatataagcaacgatcacatcgacacctgggagtggaatgatgtgacgctctacggcatgctcaacacactcaagaacaggaaccccaacctgaagactctcttgtctgtcggaggatggaactttgggtctcaaagattttccaagatagcctccaacacccagagtcgccggactttcatcaagtcagtaccgccatttctgcgcacccatggctttgatgggctggaccttgcctggctctaccctggacggagagacaaacagcattttaccaccctaatcaaggaaatgaaggccgaatttataaaggaagcccagccagggaaaaagcagctcctgctcagcgcagcactgtctgcggggaaggtcaccattgacagcagctatgacattgccaagatatcccaacacctggatttcattagcatcatgacctacgattttcatggagcctggcgtgggaccacaggccatcacagtcccctgttccgaggtcaggaggatgcaagtcctgacagattcagcaacactgactatgctgtggggtacatgttgaggctgggggctcctgccagtaagctggtgatgggcatccccaccttcgggaggagcttcactctggcttcttctgagactggtgttggagccccaatctcaggaccgggaattccaggccggttcaccaaggaggcagggacccttgcctactatgagatctgtgacttcctccgcggagccacagtccatagaatcctcggccagcaggtcccctatgccaccaagggcaaccagtgggtaggatacgacgaccaggaaagcgtcaaaagcaaggtgcagtacctgaaggacaggcagctggcgggcgccatggtatgggccctggacctggatgacttccagggctccttctgcggccaggatctgcgcttccctctcaccaatgccatcaaggatgcactcgctgcaacgtag

SEQ ID NO: 2 - protein, 383 aa, Homo sapiens
MGVKASQTGFVVLVLLQCCSAYKLVCYYTSWSQYREGDGSCFPDALDRFLCTHIIYSFANISNDHIDTWEWNDVTLYGMLNTLKNRNPNLKTLLSVGGWNFGSQRFSKIASNTQSRRTFIKSVPPFLRTHGFDGLDLAWLYPGRRDKQHFTTLIKEMKAEFIKEAQPGKKQLLLSAALSAGKVTIDSSYDIAKISQHLDFISIMTYDFHGAWRGTTGHHSPLFRGQEDASPDRFSNTDYAVGYMLRLGAPASKLVMGIPTFGRSFTLASSETGVGAPISGPGIPGRFTKEAGTLAYYEICDFLRGATVHRILGQQVPYATKGNQWVGYDDQESVKSKVQYLKDRQLAGAMVWALDLDDFQGSFCGQDLRFPLTNAIKDALAAT